European Patent Specification EP 3 795 170 B1, published March 20, 2024. Title: PHARMACEUTICAL COMPOSITION COMPRISING CCN5 AS EFFECTIVE INGREDIENT, FOR PREVENTING OR TREATING RETINAL DISEASES. Applicant: OLIVES BIOTHERAPEUTICS INC. The sequence listing filed with the application follows.

SEQUENCE LISTING (6 sequences)

SEQ ID NO: 1 - protein, 251 aa, Artificial Sequence
  CCN5(mouse)
MRGNPLIHLLAISFLCILSMVYSQLCPAPCACPWTPPQCPPGVPLVLDGCGCCRVCARRLGESCDHLHVCDPSQGLVCQPGAGPSGRGAVCLFEEDDGSCEVNGRRYLDGETFKPNCRVLCRCDDGGFTCLPLCSEDVRLPSWDCPRPRRIQVPGRCCPEWVCDQAVMQPAIQPSSAQGHQLSALVTPASADGPCPNWSTAWGPCSTTCGLGIATRVSNQNRFCQLEIQRRLCLSRPCLASRSHGSWNSAF

SEQ ID NO: 2 - DNA, 756 bp, Artificial Sequence
  CCN5(mouse)
atgaggggcaacccactgatccatcttctggccatttccttcctctgcattctctcaatggtgtatgcccagctgtgcccagcaccctgtgcctgtccttggacaccaccccagtgcccaccgggggtacccctggtgctggatggctgtggctgctgtcgagtgtgtgcacggaggctgggggagtcctgcgaccacctgcatgtctgcaaccccagccagggcctggtttgtcagcctggggcaggccccagtggccgtggtgttgtgtgcctcttcgaagaggatgacgggagctgtgaggtgaacggccgcaggtacctggatggggagacctttaaacccaattgcagggttttgtgccgctgtgatgacggtggtttcacctgcctgccgctgtgcagtgaggatgtgcggctgcccagctgggactgcccacgccccaggagaatacaggtgccaggaaggtgctgccccgagtgggtgtgtgaccaggcagtgatgcagccggcaatccagccctcctcagcccaaggacaccaactttctgcccttgtcactcctgcatctgccgatggcccctgtccaaactggagcacagcctggggcccctgctcaaccacctgtgggttgggcatagccacccgagtatccaaccagaaccgattctgccaactggagatccagcgtcgcctgtgtctgtccagaccctgcctggcatccaggagccacggctcatggaacagtgccttctag

SEQ ID NO: 3 - protein, 228 aa, Artificial Sequence
  CCN5(except signal peptide, mouse)
QLCPAPCACPWTPPQCPPGVPLVLDGCGCCRVCARRLGESCDHLHVCDPSQGLVCQPGAGPSGRGAVCLFEEDDGSCEVNGRRYLDGETFKPNCRVLCRCDDGGFTCLPLCSEDVRLPSWDCPRPRRIQVPGRCCPEWVCDQAVMQPAIQPSSAQGHQLSALVTPASADGPCPNWSTAWGPCSTTCGLGIATRVSNQNRFCQLEIQRRLCLSRPCLASRSHGSWNSAF

SEQ ID NO: 4 - protein, 250 aa, Artificial Sequence
  CCN5(human)
MRGTPKTHLLAFSLLCLLSKVRTQLCPTPCTCPWPPPRCPLGVPLVLDGCGCCRVCARRLGEPCDQLHVCDASQGLVCQPGAGPGGRGALCLLAEDDSSCEVNGRLYREGETFQPHCSIRCRCEDGGFTCVPLCSEDVRLPSWDCPHPRRVEVLGKCCPEWVCGQGGGLGTQPLPAQGPQFSGLVSSLPPGVPCPEWSTAWGPCSTTCGLGMATRVSNQNRFCRLETQRRLCLSRPCPPSRGRSPQNSAF

SEQ ID NO: 5 - DNA, 753 bp, Artificial Sequence
  CCN5(human)
atgagaggcacaccgaagacccacctcctggccttctccctcctctgcctcctctcaaaggtgcgtacccagctgtgcccgacaccatgtacctgcccctggccacctccccgatgcccgctgggagtacccctggtgctggatggctgtggctgctgccgggtatgtgcacggcggctgggggagccctgcgaccaactccacgtctgcgacgccagccagggcctggtctgccagcccggggcaggacccggtggccggggggccctgtgcctcttggcagaggacgacagcagctgtgaggtgaacggccgcctgtatcgggaaggggagaccttccagccccactgcagcatccgctgccgctgcgaggacggcggcttcacctgcgtgccgctgtgcagcgaggatgtgcggctgcccagctgggactgcccccaccccaggagggtcgaggtcctgggcaagtgctgccctgagtgggtgtgcggccaaggagggggactggggacccagccccttccagcccaaggaccccagttttctggccttgtctcttccctgccccctggtgtcccctgcccagaatggagcacggcctggggaccctgctcgaccacctgtgggctgggcatggccacccgggtgtccaaccagaaccgcttctgccgactggagacccagcgccgcctgtgcctgtccaggccctgcccaccctccaggggtcgcagtccacaaaacagtgccttctag

SEQ ID NO: 6 - protein, 227 aa, Artificial Sequence
  CCN5(except signal peptide, human)
QLCPTPCTCPWPPPRCPLGVPLVLDGCGCCRVCARRLGEPCDQLHVCDASQGLVCQPGAGPGGRGALCLLAEDDSSCEVNGRLYREGETFQPHCSIRCRCEDGGFTCVPLCSEDVRLPSWDCPHPRRVEVLGKCCPEWVCGQGGGLGTQPLPAQGPQFSGLVSSLPPGVPCPEWSTAWGPCSTTCGLGMATRVSNQNRFCRLETQRRLCLSRPCPPSRGRSPQNSAF